European Patent Specification EP 4 008 728 B1, published December 17, 2025. Title: CD70 BINDING MOLECULES AND METHODS OF USE THEREOF. Applicant: KITE PHARMA, INC. The sequence listing filed with the application follows.

SEQUENCE LISTING (97 sequences)

SEQ ID NO: 1 - protein, 193 aa, Homo sapiens
MPEEGSGCSVRRRPYGCVLRAALVPLVAGLVICLVVCIQRFAQAQQQLPLESLGWDVAELQLNHTGPQQDPRLYWQGGPALGRSFLHGPELDKGQLRIHRDGIYMVHIQVTLAICSSTTASRHHPTTLAVGICSPASRSISLLRLSFHQGCTIASQRLTPLARGDTLCTNLTGTLLPSRNTDETFFGVQWVRP

SEQ ID NO: 2 - DNA, 366 bp, Homo sapiens
  CDS (1)..(366): 8G1 VH
caagagcagctggttgagtctgggggcggcgtcgtccaacccggccggagtctgaggttgtcctgcgctgcaagcggatttacattttcatcttacggcatgcactgggttaggcaggctcctggaaaagggctggagtgggtcgcggtgacttggtacgacggctccaataagtattatggggattccgtgaaaggtcgattcacaattagcagggataactccaaaaacacactgtatctccaaatgaactccttgagggccgaggacacggccgtctattattgtgcaagagacctcctccggggcgtaaagggatatgctatggacgtgtggggtcaggggaccacagttactgtcagttca

SEQ ID NO: 3 - protein, 122 aa, Homo sapiens
QEQLVESGGGVVQPGRSLRLSCAASGFTFSSYGMHWVRQAPGKGLEWVAVTWYDGSNKYYGDSVKGRFTISRDNSKNTLYLQMNSLRAEDTAVYYCARDLLRGVKGYAMDVWGQGTTVTVSS

SEQ ID NO: 4 - DNA, 327 bp, Homo sapiens
  CDS (1)..(327): 8G1 VL
gaaatcgttctcactcagtctccgggcacactgtccctcagccccggagagcgagccactttgagctgccgggccagccagtcacttagacgcatttatttggcctggtatcagcagaaaccaggccaggcgcccaggctgctgatatacgatgtgttcgatagggccacgggtatccccgataggttctctggcggggggtccgggactgacttcaccctcactatatcacgactcgagcccgaagacttcgcagtttattattgccagcagtactccgactccccattcaccttcggccctggtaccaaagtggatattaaacgg

SEQ ID NO: 5 - protein, 109 aa, Homo sapiens
EIVLTQSPGTLSLSPGERATLSCRASQSLRRIYLAWYQQKPGQAPRLLIYDVFDRATGIPDRFSGGGSGTDFTLTISRLEPEDFAVYYCQQYSDSPFTFGPGTKVDIKR

SEQ ID NO: 6 - DNA, 360 bp, Homo sapiens
  CDS (1)..(360): 1C8 VH
caggtgcagctccaagaatctggaccgggtctcgtcaagccatcacagacactgtccctgacctgcaccgtctccggcgactctatcatttcaggcggctactattggtcctggattagacaacatccgggaaagggtcttgaatggatcggctatattttctacagcgggagtacggattacaatcctagtctcaagagccgcgttaccatttcagtggatacttcaaaaaaccagtttagcctgaagctgtcttctgtaacagctgctgacacagccgtgtactattgcgccaggagcggctacagctatgccctgtttgaccactgggggcaaggcactcttgtgacggtgtcaagt

SEQ ID NO: 7 - protein, 120 aa, Homo sapiens
QVQLQESGPGLVKPSQTLSLTCTVSGDSIISGGYYWSWIRQHPGKGLEWIGYIFYSGSTDYNPSLKSRVTISVDTSKNQFSLKLSSVTAADTAVYYCARSGYSYALFDHWGQGTLVTVSS

SEQ ID NO: 8 - DNA, 324 bp, Homo sapiens
  CDS (1)..(324): 1C8 VL
gacattcaaatgacgcagtccccaagttctctgtccgctagcgtcggcgaccgagtgaccatcagctgccgagcatcccagtttatcggtagatatttcaattggtaccagcaacaaccgggcaaagcgcccaaggtcctgatctacgctgagagcagtctgcaatccggcgtacctagcaggttctccggaagtggcagcggaaccgagttcaccctgacaattagctccttgcagcccgaggatttcgctcgctattactgtcaacagagttattcaaccccttttacattcggacagggaactaaagttgaaattaagagg

SEQ ID NO: 9 - protein, 108 aa, Homo sapiens
DIQMTQSPSSLSASVGDRVTISCRASQFIGRYFNWYQQQPGKAPKVLIYAESSLQSGVPSRFSGSGSGTEFTLTISSLQPEDFARYYCQQSYSTPFTFGQGTKVEIKR

SEQ ID NO: 10 - DNA, 354 bp, Homo sapiens
  CDS (1)..(354): 6E9 VH
caggtacacctggtgcagagcggggcggaggtcaagaaaccgggcgcatccgtacgcgtgagctgcaaggcctccggatacacttttacttcttactatctgcattgggtcaggcaggcaccgggtcagggactggagtggatgggcattgtggacccaagcggagggagtacgtcatatgatcagaagtttcaaggtaggtttaccatgacacgggacacgtcaacgagtaccgtctacatggagctcagtagtctgcggagcgaagacaccgcagtctactactgcgcacgcgattatggagactatgtctttgactattgggggcaggggacgctcgtgaccgtttcaagc

SEQ ID NO: 11 - protein, 118 aa, Homo sapiens
QVHLVQSGAEVKKPGASVRVSCKASGYTFTSYYLHWVRQAPGQGLEWMGIVDPSGGSTSYDQKFQGRFTMTRDTSTSTVYMELSSLRSEDTAVYYCARDYGDYVFDYWGQGTLVTVSS

SEQ ID NO: 12 - DNA, 333 bp, Homo sapiens
  CDS (1)..(333): 6E9 VL
caaagcgtactgacacagcccccgagtgcatccgggacccccggccaaagggttacaatcagctgctctggcagctccagtaacataggtaccaacacggtgaactggtaccagcagttgcctggcacagcgcctcagctgctcatctatatcaacaatcagcggccaagtggcgtgcccgatagattctcaggctcaaagagcggaaccagcgctagcttggcaatcagtggccttcaatccgaagacgaagccgattactattgtgcgacctgggacgatagcctgaacggccccgtcgtgggcggcgggacgaaactgacagtgttgggc

SEQ ID NO: 13 - protein, 111 aa, Homo sapiens
QSVLTQPPSASGTPGQRVTISCSGSSSNIGTNTVNWYQQLPGTAPQLLIYINNQRPSGVPDRFSGSKSGTSASLAISGLQSEDEADYYCATWDDSLNGPVVGGGTKLTVLG

SEQ ID NO: 14 - DNA, 171 bp, Homo sapiens
  CDS (1)..(171): CD28T EC/TM
cttgataatgaaaagtcaaacggaacaatcattcacgtgaagggcaagcacctctgtccgtcacccttgttccctggtccatccaagccattctgggtgttggtcgtagtgggtggagtcctcgcttgttactctctgctcgtcaccgtggcttttataatcttctgggtt

SEQ ID NO: 15 - protein, 57 aa, Homo sapiens
LDNEKSNGTIIHVKGKHLCPSPLFPGPSKPFWVLVVVGGVLACYSLLVTVAFIIFWV

SEQ ID NO: 16 - DNA, 249 bp, Homo sapiens
  CDS (1)..(249): CD8 EC/TM
ttcgtgcctgtttttctgcccgcgaaacccacaactacccccgcccctcggcccccaactcctgcaccaactatcgcttcccaacccctgtctctgagacctgaggcatgccgccccgcggcaggcggcgccgtgcacactagaggcctggacttcgcctgcgatatttatatctgggccccccttgccgggacatgcggggtactgctgctgtctctggtgattaccctctactgcaaccacagaaac

SEQ ID NO: 17 - protein, 83 aa, Homo sapiens
FVPVFLPAKPTTTPAPRPPTPAPTIASQPLSLRPEACRPAAGGAVHTRGLDFACDIYIWAPLAGTCGVLLLSLVITLYCNHRN

SEQ ID NO: 18 - DNA, 81 bp, Homo sapiens
  CDS (1)..(81): CD28T TM
ttctgggtgttggtcgtagtgggtggagtcctcgcttgttactctctgctcgtcaccgtggcttttataatcttctgggtt

SEQ ID NO: 19 - protein, 27 aa, Homo sapiens
FWVLVVVGGVLACYSLLVTVAFIIFWV

SEQ ID NO: 20 - DNA, 63 bp, Homo sapiens
  CDS (1)..(63): CD8 TM
atttatatctgggccccccttgccgggacatgcggggtactgctgctgtctctggtgattacc

SEQ ID NO: 21 - protein, 21 aa, Homo sapiens
IYIWAPLAGTCGVLLLSLVIT

SEQ ID NO: 22 - DNA, 123 bp, Homo sapiens
  CDS (1)..(123): CD28 costim
agatccaaaagaagccgcctgctccatagcgattacatgaatatgactccacgccgccctggccccacaaggaaacactaccagccttacgcaccacctagagatttcgctgcctatcggagc

SEQ ID NO: 23 - protein, 41 aa, Homo sapiens
RSKRSRLLHSDYMNMTPRRPGPTRKHYQPYAPPRDFAAYRS

SEQ ID NO: 24 - DNA, 141 bp, Homo sapiens
  CDS (1)..(141): 4-1BB costim
cgcttttccgtcgttaagcgggggagaaaaaagctgctgtacattttcaaacagccgtttatgaggccggtccaaacgactcaggaagaagacggctgctcctgccgctttcctgaggaggaggagggcgggtgcgaactg

SEQ ID NO: 25 - protein, 47 aa, Homo sapiens
RFSVVKRGRKKLLYIFKQPFMRPVQTTQEEDGCSCRFPEEEEGGCEL

SEQ ID NO: 26 - DNA, 336 bp, Homo sapiens
  CDS (1)..(336): CD3zeta
agggtgaagttttccagatctgcagatgcaccagcgtatcagcagggccagaaccaactgtataacgagctcaacctgggacgcagggaagagtatgacgttttggacaagcgcagaggacgggaccctgagatgggtggcaaaccaagacgaaaaaacccccaggagggtctctataatgagctgcagaaggataagatggctgaagcctattctgaaataggcatgaaaggagagcggagaaggggaaaagggcacgacggtttgtaccagggactcagcactgctacgaaggatacttatgacgctctccacatgcaagccctgccacctagg

SEQ ID NO: 27 - protein, 112 aa, Homo sapiens
RVKFSRSADAPAYQQGQNQLYNELNLGRREEYDVLDKRRGRDPEMGGKPRRKNPQEGLYNELQKDKMAEAYSEIGMKGERRRGKGHDGLYQGLSTATKDTYDALHMQALPPR

SEQ ID NO: 28 - protein, 21 aa, Homo sapiens
MALPVTALLLPLALLLHAARP

SEQ ID NO: 29 - DNA, 1440 bp, Homo sapiens
  CDS (1)..(1440): 8G1.1_C28T_28z
atggcactccccgtaactgctctgctgctgccgttggcattgctcctgcacgccgcacgcccgcaagagcagctggttgagtctgggggcggcgtcgtccaacccggccggagtctgaggttgtcctgcgctgcaagcggatttacattttcatcttacggcatgcactgggttaggcaggctcctggaaaagggctggagtgggtcgcggtgacttggtacgacggctccaataagtattatggggattccgtgaaaggtcgattcacaattagcagggataactccaaaaacacactgtatctccaaatgaactccttgagggccgaggacacggccgtctattattgtgcaagagacctcctccggggcgtaaagggatatgctatggacgtgtggggtcaggggaccacagttactgtcagttcaggtggcggtggcagtggcggcgggggaagtggaggcgggggctctgaaatcgttctcactcagtctccgggcacactgtccctcagccccggagagcgagccactttgagctgccgggccagccagtcacttagacgcatttatttggcctggtatcagcagaaaccaggccaggcgcccaggctgctgatatacgatgtgttcgatagggccacgggtatccccgataggttctctggcggggggtccgggactgacttcaccctcactatatcacgactcgagcccgaagacttcgcagtttattattgccagcagtactccgactccccattcaccttcggccctggtaccaaagtggatattaaacgggccgctgcccttgataatgaaaagtcaaacggaacaatcattcacgtgaagggcaagcacctctgtccgtcacccttgttccctggtccatccaagccattctgggtgttggtcgtagtgggtggagtcctcgcttgttactctctgctcgtcaccgtggcttttataatcttctgggttagatccaaaagaagccgcctgctccatagcgattacatgaatatgactccacgccgccctggccccacaaggaaacactaccagccttacgcaccacctagagatttcgctgcctatcggagcagggtgaagttttccagatctgcagatgcaccagcgtatcagcagggccagaaccaactgtataacgagctcaacctgggacgcagggaagagtatgacgttttggacaagcgcagaggacgggaccctgagatgggtggcaaaccaagacgaaaaaacccccaggagggtctctataatgagctgcagaaggataagatggctgaagcctattctgaaataggcatgaaaggagagcggagaaggggaaaagggcacgacggtttgtaccagggactcagcactgctacgaaggatacttatgacgctctccacatgcaagccctgccacctagg

SEQ ID NO: 30 - protein, 480 aa, Homo sapiens
MALPVTALLLPLALLLHAARPQEQLVESGGGVVQPGRSLRLSCAASGFTFSSYGMHWVRQAPGKGLEWVAVTWYDGSNKYYGDSVKGRFTISRDNSKNTLYLQMNSLRAEDTAVYYCARDLLRGVKGYAMDVWGQGTTVTVSSGGGGSGGGGSGGGGSEIVLTQSPGTLSLSPGERATLSCRASQSLRRIYLAWYQQKPGQAPRLLIYDVFDRATGIPDRFSGGGSGTDFTLTISRLEPEDFAVYYCQQYSDSPFTFGPGTKVDIKRAAALDNEKSNGTIIHVKGKHLCPSPLFPGPSKPFWVLVVVGGVLACYSLLVTVAFIIFWVRSKRSRLLHSDYMNMTPRRPGPTRKHYQPYAPPRDFAAYRSRVKFSRSADAPAYQQGQNQLYNELNLGRREEYDVLDKRRGRDPEMGGKPRRKNPQEGLYNELQKDKMAEAYSEIGMKGERRRGKGHDGLYQGLSTATKDTYDALHMQALPPR

SEQ ID NO: 31 - DNA, 1458 bp, Homo sapiens
  CDS (1)..(1458): 8G1.1_C28T_4Bz
atggcactccccgtaactgctctgctgctgccgttggcattgctcctgcacgccgcacgcccgcaagagcagctggttgagtctgggggcggcgtcgtccaacccggccggagtctgaggttgtcctgcgctgcaagcggatttacattttcatcttacggcatgcactgggttaggcaggctcctggaaaagggctggagtgggtcgcggtgacttggtacgacggctccaataagtattatggggattccgtgaaaggtcgattcacaattagcagggataactccaaaaacacactgtatctccaaatgaactccttgagggccgaggacacggccgtctattattgtgcaagagacctcctccggggcgtaaagggatatgctatggacgtgtggggtcaggggaccacagttactgtcagttcaggtggcggtggcagtggcggcgggggaagtggaggcgggggctctgaaatcgttctcactcagtctccgggcacactgtccctcagccccggagagcgagccactttgagctgccgggccagccagtcacttagacgcatttatttggcctggtatcagcagaaaccaggccaggcgcccaggctgctgatatacgatgtgttcgatagggccacgggtatccccgataggttctctggcggggggtccgggactgacttcaccctcactatatcacgactcgagcccgaagacttcgcagtttattattgccagcagtactccgactccccattcaccttcggccctggtaccaaagtggatattaaacgggccgctgcccttgataatgaaaagtcaaacggaacaatcattcacgtgaagggcaagcacctctgtccgtcacccttgttccctggtccatccaagccattctgggtgttggtcgtagtgggtggagtcctcgcttgttactctctgctcgtcaccgtggcttttataatcttctgggttcgcttttccgtcgttaagcgggggagaaaaaagctgctgtacattttcaaacagccgtttatgaggccggtccaaacgactcaggaagaagacggctgctcctgccgctttcctgaggaggaggagggcgggtgcgaactgagggtgaagttttccagatctgcagatgcaccagcgtatcagcagggccagaaccaactgtataacgagctcaacctgggacgcagggaagagtatgacgttttggacaagcgcagaggacgggaccctgagatgggtggcaaaccaagacgaaaaaacccccaggagggtctctataatgagctgcagaaggataagatggctgaagcctattctgaaataggcatgaaaggagagcggagaaggggaaaagggcacgacggtttgtaccagggactcagcactgctacgaaggatacttatgacgctctccacatgcaagccctgccacctagg

SEQ ID NO: 32 - protein, 486 aa, Homo sapiens
MALPVTALLLPLALLLHAARPQEQLVESGGGVVQPGRSLRLSCAASGFTFSSYGMHWVRQAPGKGLEWVAVTWYDGSNKYYGDSVKGRFTISRDNSKNTLYLQMNSLRAEDTAVYYCARDLLRGVKGYAMDVWGQGTTVTVSSGGGGSGGGGSGGGGSEIVLTQSPGTLSLSPGERATLSCRASQSLRRIYLAWYQQKPGQAPRLLIYDVFDRATGIPDRFSGGGSGTDFTLTISRLEPEDFAVYYCQQYSDSPFTFGPGTKVDIKRAAALDNEKSNGTIIHVKGKHLCPSPLFPGPSKPFWVLVVVGGVLACYSLLVTVAFIIFWVRFSVVKRGRKKLLYIFKQPFMRPVQTTQEEDGCSCRFPEEEEGGCELRVKFSRSADAPAYQQGQNQLYNELNLGRREEYDVLDKRRGRDPEMGGKPRRKNPQEGLYNELQKDKMAEAYSEIGMKGERRRGKGHDGLYQGLSTATKDTYDALHMQALPPR

SEQ ID NO: 33 - DNA, 1518 bp, Homo sapiens
  CDS (1)..(1518): 8G1.1_C8K_28z
atggcactccccgtaactgctctgctgctgccgttggcattgctcctgcacgccgcacgcccgcaagagcagctggttgagtctgggggcggcgtcgtccaacccggccggagtctgaggttgtcctgcgctgcaagcggatttacattttcatcttacggcatgcactgggttaggcaggctcctggaaaagggctggagtgggtcgcggtgacttggtacgacggctccaataagtattatggggattccgtgaaaggtcgattcacaattagcagggataactccaaaaacacactgtatctccaaatgaactccttgagggccgaggacacggccgtctattattgtgcaagagacctcctccggggcgtaaagggatatgctatggacgtgtggggtcaggggaccacagttactgtcagttcaggtggcggtggcagtggcggcgggggaagtggaggcgggggctctgaaatcgttctcactcagtctccgggcacactgtccctcagccccggagagcgagccactttgagctgccgggccagccagtcacttagacgcatttatttggcctggtatcagcagaaaccaggccaggcgcccaggctgctgatatacgatgtgttcgatagggccacgggtatccccgataggttctctggcggggggtccgggactgacttcaccctcactatatcacgactcgagcccgaagacttcgcagtttattattgccagcagtactccgactccccattcaccttcggccctggtaccaaagtggatattaaacgggccgctgccttcgtgcctgtttttctgcccgcgaaacccacaactacccccgcccctcggcccccaactcctgcaccaactatcgcttcccaacccctgtctctgagacctgaggcatgccgccccgcggcaggcggcgccgtgcacactagaggcctggacttcgcctgcgatatttatatctgggccccccttgccgggacatgcggggtactgctgctgtctctggtgattaccctctactgcaaccacagaaacagatccaaaagaagccgcctgctccatagcgattacatgaatatgactccacgccgccctggccccacaaggaaacactaccagccttacgcaccacctagagatttcgctgcctatcggagcagggtgaagttttccagatctgcagatgcaccagcgtatcagcagggccagaaccaactgtataacgagctcaacctgggacgcagggaagagtatgacgttttggacaagcgcagaggacgggaccctgagatgggtggcaaaccaagacgaaaaaacccccaggagggtctctataatgagctgcagaaggataagatggctgaagcctattctgaaataggcatgaaaggagagcggagaaggggaaaagggcacgacggtttgtaccagggactcagcactgctacgaaggatacttatgacgctctccacatgcaagccctgccacctagg

SEQ ID NO: 34 - protein, 506 aa, Homo sapiens
MALPVTALLLPLALLLHAARPQEQLVESGGGVVQPGRSLRLSCAASGFTFSSYGMHWVRQAPGKGLEWVAVTWYDGSNKYYGDSVKGRFTISRDNSKNTLYLQMNSLRAEDTAVYYCARDLLRGVKGYAMDVWGQGTTVTVSSGGGGSGGGGSGGGGSEIVLTQSPGTLSLSPGERATLSCRASQSLRRIYLAWYQQKPGQAPRLLIYDVFDRATGIPDRFSGGGSGTDFTLTISRLEPEDFAVYYCQQYSDSPFTFGPGTKVDIKRAAAFVPVFLPAKPTTTPAPRPPTPAPTIASQPLSLRPEACRPAAGGAVHTRGLDFACDIYIWAPLAGTCGVLLLSLVITLYCNHRNRSKRSRLLHSDYMNMTPRRPGPTRKHYQPYAPPRDFAAYRSRVKFSRSADAPAYQQGQNQLYNELNLGRREEYDVLDKRRGRDPEMGGKPRRKNPQEGLYNELQKDKMAEAYSEIGMKGERRRGKGHDGLYQGLSTATKDTYDALHMQALPPR

SEQ ID NO: 35 - DNA, 1056 bp, Homo sapiens
  CDS (1)..(1056): 8G1.1_C8K_4Bz
gttctcactcagtctccgggcacactgtccctcagccccggagagcgagccactttgagctgccgggccagccagtcacttagacgcatttatttggcctggtatcagcagaaaccaggccaggcgcccaggctgctgatatacgatgtgttcgatagggccacgggtatccccgataggttctctggcggggggtccgggactgacttcaccctcactatatcacgactcgagcccgaagacttcgcagtttattattgccagcagtactccgactccccattcaccttcggccctggtaccaaagtggatattaaacgggccgctgccttcgtgcctgtttttctgcccgcgaaacccacaactacccccgcccctcggcccccaactcctgcaccaactatcgcttcccaacccctgtctctgagacctgaggcatgccgccccgcggcaggcggcgccgtgcacactagaggcctggacttcgcctgcgatatttatatctgggccccccttgccgggacatgcggggtactgctgctgtctctggtgattaccctctactgcaaccacagaaaccgcttttccgtcgttaagcgggggagaaaaaagctgctgtacattttcaaacagccgtttatgaggccggtccaaacgactcaggaagaagacggctgctcctgccgctttcctgaggaggaggagggcgggtgcgaactgagggtgaagttttccagatctgcagatgcaccagcgtatcagcagggccagaaccaactgtataacgagctcaacctgggacgcagggaagagtatgacgttttggacaagcgcagaggacgggaccctgagatgggtggcaaaccaagacgaaaaaacccccaggagggtctctataatgagctgcagaaggataagatggctgaagcctattctgaaataggcatgaaaggagagcggagaaggggaaaagggcacgacggtttgtaccagggactcagcactgctacgaaggatacttatgacgctctccacatgcaagccctgccacctagg

SEQ ID NO: 36 - protein, 352 aa, Homo sapiens
VLTQSPGTLSLSPGERATLSCRASQSLRRIYLAWYQQKPGQAPRLLIYDVFDRATGIPDRFSGGGSGTDFTLTISRLEPEDFAVYYCQQYSDSPFTFGPGTKVDIKRAAAFVPVFLPAKPTTTPAPRPPTPAPTIASQPLSLRPEACRPAAGGAVHTRGLDFACDIYIWAPLAGTCGVLLLSLVITLYCNHRNRFSVVKRGRKKLLYIFKQPFMRPVQTTQEEDGCSCRFPEEEEGGCELRVKFSRSADAPAYQQGQNQLYNELNLGRREEYDVLDKRRGRDPEMGGKPRRKNPQEGLYNELQKDKMAEAYSEIGMKGERRRGKGHDGLYQGLSTATKDTYDALHMQALPPR

SEQ ID NO: 37 - DNA, 1431 bp, Homo sapiens
  CDS (1)..(1431): 1C8.1.001_C28T_28z
atggcactccccgtaactgctctgctgctgccgttggcattgctcctgcacgccgcacgcccgcaggtgcagctccaagaatctggaccgggtctcgtcaagccatcacagacactgtccctgacctgcaccgtctccggcgactctatcatttcaggcggctactattggtcctggattagacaacatccgggaaagggtcttgaatggatcggctatattttctacagcgggagtacggattacaatcctagtctcaagagccgcgttaccatttcagtggatacttcaaaaaaccagtttagcctgaagctgtcttctgtaacagctgctgacacagccgtgtactattgcgccaggagcggctacagctatgccctgtttgaccactgggggcaaggcactcttgtgacggtgtcaagtggagggggaggatcaggcggcgggggatccggcggcgggggtagtgacattcaaatgacgcagtccccaagttctctgtccgctagcgtcggcgaccgagtgaccatcagctgccgagcatcccagtttatcggtagatatttcaattggtaccagcaacaaccgggcaaagcgcccaaggtcctgatctacgctgagagcagtctgcaatccggcgtacctagcaggttctccggaagtggcagcggaaccgagttcaccctgacaattagctccttgcagcccgaggatttcgctcgctattactgtcaacagagttattcaaccccttttacattcggacagggaactaaagttgaaattaagagggccgctgcccttgataatgaaaagtcaaacggaacaatcattcacgtgaagggcaagcacctctgtccgtcacccttgttccctggtccatccaagccattctgggtgttggtcgtagtgggtggagtcctcgcttgttactctctgctcgtcaccgtggcttttataatcttctgggttagatccaaaagaagccgcctgctccatagcgattacatgaatatgactccacgccgccctggccccacaaggaaacactaccagccttacgcaccacctagagatttcgctgcctatcggagcagggtgaagttttccagatctgcagatgcaccagcgtatcagcagggccagaaccaactgtataacgagctcaacctgggacgcagggaagagtatgacgttttggacaagcgcagaggacgggaccctgagatgggtggcaaaccaagacgaaaaaacccccaggagggtctctataatgagctgcagaaggataagatggctgaagcctattctgaaataggcatgaaaggagagcggagaaggggaaaagggcacgacggtttgtaccagggactcagcactgctacgaaggatacttatgacgctctccacatgcaagccctgccacctagg

SEQ ID NO: 38 - protein, 477 aa, Homo sapiens
MALPVTALLLPLALLLHAARPQVQLQESGPGLVKPSQTLSLTCTVSGDSIISGGYYWSWIRQHPGKGLEWIGYIFYSGSTDYNPSLKSRVTISVDTSKNQFSLKLSSVTAADTAVYYCARSGYSYALFDHWGQGTLVTVSSGGGGSGGGGSGGGGSDIQMTQSPSSLSASVGDRVTISCRASQFIGRYFNWYQQQPGKAPKVLIYAESSLQSGVPSRFSGSGSGTEFTLTISSLQPEDFARYYCQQSYSTPFTFGQGTKVEIKRAAALDNEKSNGTIIHVKGKHLCPSPLFPGPSKPFWVLVVVGGVLACYSLLVTVAFIIFWVRSKRSRLLHSDYMNMTPRRPGPTRKHYQPYAPPRDFAAYRSRVKFSRSADAPAYQQGQNQLYNELNLGRREEYDVLDKRRGRDPEMGGKPRRKNPQEGLYNELQKDKMAEAYSEIGMKGERRRGKGHDGLYQGLSTATKDTYDALHMQALPPR

SEQ ID NO: 39 - DNA, 1449 bp, Homo sapiens
  CDS (1)..(1449): 1C8.1.001_C28T_4Bz
atggcactccccgtaactgctctgctgctgccgttggcattgctcctgcacgccgcacgcccgcaggtgcagctccaagaatctggaccgggtctcgtcaagccatcacagacactgtccctgacctgcaccgtctccggcgactctatcatttcaggcggctactattggtcctggattagacaacatccgggaaagggtcttgaatggatcggctatattttctacagcgggagtacggattacaatcctagtctcaagagccgcgttaccatttcagtggatacttcaaaaaaccagtttagcctgaagctgtcttctgtaacagctgctgacacagccgtgtactattgcgccaggagcggctacagctatgccctgtttgaccactgggggcaaggcactcttgtgacggtgtcaagtggagggggaggatcaggcggcgggggatccggcggcgggggtagtgacattcaaatgacgcagtccccaagttctctgtccgctagcgtcggcgaccgagtgaccatcagctgccgagcatcccagtttatcggtagatatttcaattggtaccagcaacaaccgggcaaagcgcccaaggtcctgatctacgctgagagcagtctgcaatccggcgtacctagcaggttctccggaagtggcagcggaaccgagttcaccctgacaattagctccttgcagcccgaggatttcgctcgctattactgtcaacagagttattcaaccccttttacattcggacagggaactaaagttgaaattaagagggccgctgcccttgataatgaaaagtcaaacggaacaatcattcacgtgaagggcaagcacctctgtccgtcacccttgttccctggtccatccaagccattctgggtgttggtcgtagtgggtggagtcctcgcttgttactctctgctcgtcaccgtggcttttataatcttctgggttcgcttttccgtcgttaagcgggggagaaaaaagctgctgtacattttcaaacagccgtttatgaggccggtccaaacgactcaggaagaagacggctgctcctgccgctttcctgaggaggaggagggcgggtgcgaactgagggtgaagttttccagatctgcagatgcaccagcgtatcagcagggccagaaccaactgtataacgagctcaacctgggacgcagggaagagtatgacgttttggacaagcgcagaggacgggaccctgagatgggtggcaaaccaagacgaaaaaacccccaggagggtctctataatgagctgcagaaggataagatggctgaagcctattctgaaataggcatgaaaggagagcggagaaggggaaaagggcacgacggtttgtaccagggactcagcactgctacgaaggatacttatgacgctctccacatgcaagccctgccacctagg

SEQ ID NO: 40 - protein, 483 aa, Homo sapiens
MALPVTALLLPLALLLHAARPQVQLQESGPGLVKPSQTLSLTCTVSGDSIISGGYYWSWIRQHPGKGLEWIGYIFYSGSTDYNPSLKSRVTISVDTSKNQFSLKLSSVTAADTAVYYCARSGYSYALFDHWGQGTLVTVSSGGGGSGGGGSGGGGSDIQMTQSPSSLSASVGDRVTISCRASQFIGRYFNWYQQQPGKAPKVLIYAESSLQSGVPSRFSGSGSGTEFTLTISSLQPEDFARYYCQQSYSTPFTFGQGTKVEIKRAAALDNEKSNGTIIHVKGKHLCPSPLFPGPSKPFWVLVVVGGVLACYSLLVTVAFIIFWVRFSVVKRGRKKLLYIFKQPFMRPVQTTQEEDGCSCRFPEEEEGGCELRVKFSRSADAPAYQQGQNQLYNELNLGRREEYDVLDKRRGRDPEMGGKPRRKNPQEGLYNELQKDKMAEAYSEIGMKGERRRGKGHDGLYQGLSTATKDTYDALHMQALPPR

SEQ ID NO: 41 - DNA, 1509 bp, Homo sapiens
  CDS (1)..(1509): 1C8.1.001_C8K_28z
atggcactccccgtaactgctctgctgctgccgttggcattgctcctgcacgccgcacgcccgcaggtgcagctccaagaatctggaccgggtctcgtcaagccatcacagacactgtccctgacctgcaccgtctccggcgactctatcatttcaggcggctactattggtcctggattagacaacatccgggaaagggtcttgaatggatcggctatattttctacagcgggagtacggattacaatcctagtctcaagagccgcgttaccatttcagtggatacttcaaaaaaccagtttagcctgaagctgtcttctgtaacagctgctgacacagccgtgtactattgcgccaggagcggctacagctatgccctgtttgaccactgggggcaaggcactcttgtgacggtgtcaagtggagggggaggatcaggcggcgggggatccggcggcgggggtagtgacattcaaatgacgcagtccccaagttctctgtccgctagcgtcggcgaccgagtgaccatcagctgccgagcatcccagtttatcggtagatatttcaattggtaccagcaacaaccgggcaaagcgcccaaggtcctgatctacgctgagagcagtctgcaatccggcgtacctagcaggttctccggaagtggcagcggaaccgagttcaccctgacaattagctccttgcagcccgaggatttcgctcgctattactgtcaacagagttattcaaccccttttacattcggacagggaactaaagttgaaattaagagggccgctgccttcgtgcctgtttttctgcccgcgaaacccacaactacccccgcccctcggcccccaactcctgcaccaactatcgcttcccaacccctgtctctgagacctgaggcatgccgccccgcggcaggcggcgccgtgcacactagaggcctggacttcgcctgcgatatttatatctgggccccccttgccgggacatgcggggtactgctgctgtctctggtgattaccctctactgcaaccacagaaacagatccaaaagaagccgcctgctccatagcgattacatgaatatgactccacgccgccctggccccacaaggaaacactaccagccttacgcaccacctagagatttcgctgcctatcggagcagggtgaagttttccagatctgcagatgcaccagcgtatcagcagggccagaaccaactgtataacgagctcaacctgggacgcagggaagagtatgacgttttggacaagcgcagaggacgggaccctgagatgggtggcaaaccaagacgaaaaaacccccaggagggtctctataatgagctgcagaaggataagatggctgaagcctattctgaaataggcatgaaaggagagcggagaaggggaaaagggcacgacggtttgtaccagggactcagcactgctacgaaggatacttatgacgctctccacatgcaagccctgccacctagg

SEQ ID NO: 42 - protein, 503 aa, Homo sapiens
MALPVTALLLPLALLLHAARPQVQLQESGPGLVKPSQTLSLTCTVSGDSIISGGYYWSWIRQHPGKGLEWIGYIFYSGSTDYNPSLKSRVTISVDTSKNQFSLKLSSVTAADTAVYYCARSGYSYALFDHWGQGTLVTVSSGGGGSGGGGSGGGGSDIQMTQSPSSLSASVGDRVTISCRASQFIGRYFNWYQQQPGKAPKVLIYAESSLQSGVPSRFSGSGSGTEFTLTISSLQPEDFARYYCQQSYSTPFTFGQGTKVEIKRAAAFVPVFLPAKPTTTPAPRPPTPAPTIASQPLSLRPEACRPAAGGAVHTRGLDFACDIYIWAPLAGTCGVLLLSLVITLYCNHRNRSKRSRLLHSDYMNMTPRRPGPTRKHYQPYAPPRDFAAYRSRVKFSRSADAPAYQQGQNQLYNELNLGRREEYDVLDKRRGRDPEMGGKPRRKNPQEGLYNELQKDKMAEAYSEIGMKGERRRGKGHDGLYQGLSTATKDTYDALHMQALPPR

SEQ ID NO: 43 - DNA, 1527 bp, Homo sapiens
  CDS (1)..(1527): 1C8.1.001_C8K_4Bz
atggcactccccgtaactgctctgctgctgccgttggcattgctcctgcacgccgcacgcccgcaggtgcagctccaagaatctggaccgggtctcgtcaagccatcacagacactgtccctgacctgcaccgtctccggcgactctatcatttcaggcggctactattggtcctggattagacaacatccgggaaagggtcttgaatggatcggctatattttctacagcgggagtacggattacaatcctagtctcaagagccgcgttaccatttcagtggatacttcaaaaaaccagtttagcctgaagctgtcttctgtaacagctgctgacacagccgtgtactattgcgccaggagcggctacagctatgccctgtttgaccactgggggcaaggcactcttgtgacggtgtcaagtggagggggaggatcaggcggcgggggatccggcggcgggggtagtgacattcaaatgacgcagtccccaagttctctgtccgctagcgtcggcgaccgagtgaccatcagctgccgagcatcccagtttatcggtagatatttcaattggtaccagcaacaaccgggcaaagcgcccaaggtcctgatctacgctgagagcagtctgcaatccggcgtacctagcaggttctccggaagtggcagcggaaccgagttcaccctgacaattagctccttgcagcccgaggatttcgctcgctattactgtcaacagagttattcaaccccttttacattcggacagggaactaaagttgaaattaagagggccgctgccttcgtgcctgtttttctgcccgcgaaacccacaactacccccgcccctcggcccccaactcctgcaccaactatcgcttcccaacccctgtctctgagacctgaggcatgccgccccgcggcaggcggcgccgtgcacactagaggcctggacttcgcctgcgatatttatatctgggccccccttgccgggacatgcggggtactgctgctgtctctggtgattaccctctactgcaaccacagaaaccgcttttccgtcgttaagcgggggagaaaaaagctgctgtacattttcaaacagccgtttatgaggccggtccaaacgactcaggaagaagacggctgctcctgccgctttcctgaggaggaggagggcgggtgcgaactgagggtgaagttttccagatctgcagatgcaccagcgtatcagcagggccagaaccaactgtataacgagctcaacctgggacgcagggaagagtatgacgttttggacaagcgcagaggacgggaccctgagatgggtggcaaaccaagacgaaaaaacccccaggagggtctctataatgagctgcagaaggataagatggctgaagcctattctgaaataggcatgaaaggagagcggagaaggggaaaagggcacgacggtttgtaccagggactcagcactgctacgaaggatacttatgacgctctccacatgcaagccctgccacctagg

SEQ ID NO: 44 - protein, 509 aa, Homo sapiens
MALPVTALLLPLALLLHAARPQVQLQESGPGLVKPSQTLSLTCTVSGDSIISGGYYWSWIRQHPGKGLEWIGYIFYSGSTDYNPSLKSRVTISVDTSKNQFSLKLSSVTAADTAVYYCARSGYSYALFDHWGQGTLVTVSSGGGGSGGGGSGGGGSDIQMTQSPSSLSASVGDRVTISCRASQFIGRYFNWYQQQPGKAPKVLIYAESSLQSGVPSRFSGSGSGTEFTLTISSLQPEDFARYYCQQSYSTPFTFGQGTKVEIKRAAAFVPVFLPAKPTTTPAPRPPTPAPTIASQPLSLRPEACRPAAGGAVHTRGLDFACDIYIWAPLAGTCGVLLLSLVITLYCNHRNRFSVVKRGRKKLLYIFKQPFMRPVQTTQEEDGCSCRFPEEEEGGCELRVKFSRSADAPAYQQGQNQLYNELNLGRREEYDVLDKRRGRDPEMGGKPRRKNPQEGLYNELQKDKMAEAYSEIGMKGERRRGKGHDGLYQGLSTATKDTYDALHMQALPPR

SEQ ID NO: 45 - DNA, 1434 bp, Homo sapiens
  CDS (1)..(1434): 6E9.1_C28T_28z
atggcactccccgtaactgctctgctgctgccgttggcattgctcctgcacgccgcacgcccgcaggtacacctggtgcagagcggggcggaggtcaagaaaccgggcgcatccgtacgcgtgagctgcaaggcctccggatacacttttacttcttactatctgcattgggtcaggcaggcaccgggtcagggactggagtggatgggcattgtggacccaagcggagggagtacgtcatatgatcagaagtttcaaggtaggtttaccatgacacgggacacgtcaacgagtaccgtctacatggagctcagtagtctgcggagcgaagacaccgcagtctactactgcgcacgcgattatggagactatgtctttgactattgggggcaggggacgctcgtgaccgtttcaagcggggggggcggatccggtgggggaggttccggcggtgggggttcacaaagcgtactgacacagcccccgagtgcatccgggacccccggccaaagggttacaatcagctgctctggcagctccagtaacataggtaccaacacggtgaactggtaccagcagttgcctggcacagcgcctcagctgctcatctatatcaacaatcagcggccaagtggcgtgcccgatagattctcaggctcaaagagcggaaccagcgctagcttggcaatcagtggccttcaatccgaagacgaagccgattactattgtgcgacctgggacgatagcctgaacggccccgtcgtgggcggcgggacgaaactgacagtgttgggcgccgctgcccttgataatgaaaagtcaaacggaacaatcattcacgtgaagggcaagcacctctgtccgtcacccttgttccctggtccatccaagccattctgggtgttggtcgtagtgggtggagtcctcgcttgttactctctgctcgtcaccgtggcttttataatcttctgggttagatccaaaagaagccgcctgctccatagcgattacatgaatatgactccacgccgccctggccccacaaggaaacactaccagccttacgcaccacctagagatttcgctgcctatcggagcagggtgaagttttccagatctgcagatgcaccagcgtatcagcagggccagaaccaactgtataacgagctcaacctgggacgcagggaagagtatgacgttttggacaagcgcagaggacgggaccctgagatgggtggcaaaccaagacgaaaaaacccccaggagggtctctataatgagctgcagaaggataagatggctgaagcctattctgaaataggcatgaaaggagagcggagaaggggaaaagggcacgacggtttgtaccagggactcagcactgctacgaaggatacttatgacgctctccacatgcaagccctgccacctagg

SEQ ID NO: 46 - protein, 478 aa, Homo sapiens
MALPVTALLLPLALLLHAARPQVHLVQSGAEVKKPGASVRVSCKASGYTFTSYYLHWVRQAPGQGLEWMGIVDPSGGSTSYDQKFQGRFTMTRDTSTSTVYMELSSLRSEDTAVYYCARDYGDYVFDYWGQGTLVTVSSGGGGSGGGGSGGGGSQSVLTQPPSASGTPGQRVTISCSGSSSNIGTNTVNWYQQLPGTAPQLLIYINNQRPSGVPDRFSGSKSGTSASLAISGLQSEDEADYYCATWDDSLNGPVVGGGTKLTVLGAAALDNEKSNGTIIHVKGKHLCPSPLFPGPSKPFWVLVVVGGVLACYSLLVTVAFIIFWVRSKRSRLLHSDYMNMTPRRPGPTRKHYQPYAPPRDFAAYRSRVKFSRSADAPAYQQGQNQLYNELNLGRREEYDVLDKRRGRDPEMGGKPRRKNPQEGLYNELQKDKMAEAYSEIGMKGERRRGKGHDGLYQGLSTATKDTYDALHMQALPPR

SEQ ID NO: 47 - DNA, 1452 bp, Homo sapiens
  CDS (1)..(1452): 6E9.1_C28T_4Bz
atggcactccccgtaactgctctgctgctgccgttggcattgctcctgcacgccgcacgcccgcaggtacacctggtgcagagcggggcggaggtcaagaaaccgggcgcatccgtacgcgtgagctgcaaggcctccggatacacttttacttcttactatctgcattgggtcaggcaggcaccgggtcagggactggagtggatgggcattgtggacccaagcggagggagtacgtcatatgatcagaagtttcaaggtaggtttaccatgacacgggacacgtcaacgagtaccgtctacatggagctcagtagtctgcggagcgaagacaccgcagtctactactgcgcacgcgattatggagactatgtctttgactattgggggcaggggacgctcgtgaccgtttcaagcggggggggcggatccggtgggggaggttccggcggtgggggttcacaaagcgtactgacacagcccccgagtgcatccgggacccccggccaaagggttacaatcagctgctctggcagctccagtaacataggtaccaacacggtgaactggtaccagcagttgcctggcacagcgcctcagctgctcatctatatcaacaatcagcggccaagtggcgtgcccgatagattctcaggctcaaagagcggaaccagcgctagcttggcaatcagtggccttcaatccgaagacgaagccgattactattgtgcgacctgggacgatagcctgaacggccccgtcgtgggcggcgggacgaaactgacagtgttgggcgccgctgcccttgataatgaaaagtcaaacggaacaatcattcacgtgaagggcaagcacctctgtccgtcacccttgttccctggtccatccaagccattctgggtgttggtcgtagtgggtggagtcctcgcttgttactctctgctcgtcaccgtggcttttataatcttctgggttcgcttttccgtcgttaagcgggggagaaaaaagctgctgtacattttcaaacagccgtttatgaggccggtccaaacgactcaggaagaagacggctgctcctgccgctttcctgaggaggaggagggcgggtgcgaactgagggtgaagttttccagatctgcagatgcaccagcgtatcagcagggccagaaccaactgtataacgagctcaacctgggacgcagggaagagtatgacgttttggacaagcgcagaggacgggaccctgagatgggtggcaaaccaagacgaaaaaacccccaggagggtctctataatgagctgcagaaggataagatggctgaagcctattctgaaataggcatgaaaggagagcggagaaggggaaaagggcacgacggtttgtaccagggactcagcactgctacgaaggatacttatgacgctctccacatgcaagccctgccacctagg

SEQ ID NO: 48 - protein, 484 aa, Homo sapiens
MALPVTALLLPLALLLHAARPQVHLVQSGAEVKKPGASVRVSCKASGYTFTSYYLHWVRQAPGQGLEWMGIVDPSGGSTSYDQKFQGRFTMTRDTSTSTVYMELSSLRSEDTAVYYCARDYGDYVFDYWGQGTLVTVSSGGGGSGGGGSGGGGSQSVLTQPPSASGTPGQRVTISCSGSSSNIGTNTVNWYQQLPGTAPQLLIYINNQRPSGVPDRFSGSKSGTSASLAISGLQSEDEADYYCATWDDSLNGPVVGGGTKLTVLGAAALDNEKSNGTIIHVKGKHLCPSPLFPGPSKPFWVLVVVGGVLACYSLLVTVAFIIFWVRFSVVKRGRKKLLYIFKQPFMRPVQTTQEEDGCSCRFPEEEEGGCELRVKFSRSADAPAYQQGQNQLYNELNLGRREEYDVLDKRRGRDPEMGGKPRRKNPQEGLYNELQKDKMAEAYSEIGMKGERRRGKGHDGLYQGLSTATKDTYDALHMQALPPR

SEQ ID NO: 49 - DNA, 1452 bp, Homo sapiens; identical to SEQ ID NO: 47
  CDS (1)..(1452): 6E9.1_C8K_28z

SEQ ID NO: 50 - protein, 484 aa, Homo sapiens; identical to SEQ ID NO: 48

SEQ ID NO: 51 - DNA, 1530 bp, Homo sapiens
  CDS (1)..(1530): 6E9.1_C8K_4Bz
atggcactccccgtaactgctctgctgctgccgttggcattgctcctgcacgccgcacgcccgcaggtacacctggtgcagagcggggcggaggtcaagaaaccgggcgcatccgtacgcgtgagctgcaaggcctccggatacacttttacttcttactatctgcattgggtcaggcaggcaccgggtcagggactggagtggatgggcattgtggacccaagcggagggagtacgtcatatgatcagaagtttcaaggtaggtttaccatgacacgggacacgtcaacgagtaccgtctacatggagctcagtagtctgcggagcgaagacaccgcagtctactactgcgcacgcgattatggagactatgtctttgactattgggggcaggggacgctcgtgaccgtttcaagcggggggggcggatccggtgggggaggttccggcggtgggggttcacaaagcgtactgacacagcccccgagtgcatccgggacccccggccaaagggttacaatcagctgctctggcagctccagtaacataggtaccaacacggtgaactggtaccagcagttgcctggcacagcgcctcagctgctcatctatatcaacaatcagcggccaagtggcgtgcccgatagattctcaggctcaaagagcggaaccagcgctagcttggcaatcagtggccttcaatccgaagacgaagccgattactattgtgcgacctgggacgatagcctgaacggccccgtcgtgggcggcgggacgaaactgacagtgttgggcgccgctgccttcgtgcctgtttttctgcccgcgaaacccacaactacccccgcccctcggcccccaactcctgcaccaactatcgcttcccaacccctgtctctgagacctgaggcatgccgccccgcggcaggcggcgccgtgcacactagaggcctggacttcgcctgcgatatttatatctgggccccccttgccgggacatgcggggtactgctgctgtctctggtgattaccctctactgcaaccacagaaaccgcttttccgtcgttaagcgggggagaaaaaagctgctgtacattttcaaacagccgtttatgaggccggtccaaacgactcaggaagaagacggctgctcctgccgctttcctgaggaggaggagggcgggtgcgaactgagggtgaagttttccagatctgcagatgcaccagcgtatcagcagggccagaaccaactgtataacgagctcaacctgggacgcagggaagagtatgacgttttggacaagcgcagaggacgggaccctgagatgggtggcaaaccaagacgaaaaaacccccaggagggtctctataatgagctgcagaaggataagatggctgaagcctattctgaaataggcatgaaaggagagcggagaaggggaaaagggcacgacggtttgtaccagggactcagcactgctacgaaggatacttatgacgctctccacatgcaagccctgccacctagg

SEQ ID NO: 52 - protein, 510 aa, Homo sapiens
MALPVTALLLPLALLLHAARPQVHLVQSGAEVKKPGASVRVSCKASGYTFTSYYLHWVRQAPGQGLEWMGIVDPSGGSTSYDQKFQGRFTMTRDTSTSTVYMELSSLRSEDTAVYYCARDYGDYVFDYWGQGTLVTVSSGGGGSGGGGSGGGGSQSVLTQPPSASGTPGQRVTISCSGSSSNIGTNTVNWYQQLPGTAPQLLIYINNQRPSGVPDRFSGSKSGTSASLAISGLQSEDEADYYCATWDDSLNGPVVGGGTKLTVLGAAAFVPVFLPAKPTTTPAPRPPTPAPTIASQPLSLRPEACRPAAGGAVHTRGLDFACDIYIWAPLAGTCGVLLLSLVITLYCNHRNRFSVVKRGRKKLLYIFKQPFMRPVQTTQEEDGCSCRFPEEEEGGCELRVKFSRSADAPAYQQGQNQLYNELNLGRREEYDVLDKRRGRDPEMGGKPRRKNPQEGLYNELQKDKMAEAYSEIGMKGERRRGKGHDGLYQGLSTATKDTYDALHMQALPPR

SEQ ID NO: 53 - protein, 12 aa, Homo sapiens
RASQSLRRIYLA

SEQ ID NO: 54 - protein, 7 aa, Homo sapiens
DVFDRAT

SEQ ID NO: 55 - protein, 9 aa, Homo sapiens
QQYSDSPFT

SEQ ID NO: 56 - protein, 11 aa, Homo sapiens
RASQFIGRYFN

SEQ ID NO: 57 - protein, 7 aa, Artificial Sequence
  Description of Artificial Sequence: Synthetic peptide
AESSLQS

SEQ ID NO: 58 - protein, 9 aa, Artificial Sequence
  Description of Artificial Sequence: Synthetic peptide
QQSYSTPFT

SEQ ID NO: 59 - protein, 13 aa, Homo sapiens
SGSSSNIGTNTVN

SEQ ID NO: 60 - protein, 7 aa, Homo sapiens
INNQRPS

SEQ ID NO: 61 - protein, 12 aa, Homo sapiens
ATWDDSLNGPVV

SEQ ID NO: 62 - protein, 5 aa, Homo sapiens
SYGMH

SEQ ID NO: 63 - protein, 17 aa, Homo sapiens
VTWYDGSNKYYGDSVKG

SEQ ID NO: 64 - protein, 13 aa, Homo sapiens
DLLRGVKGYAMDV

SEQ ID NO: 65 - protein, 7 aa, Homo sapiens
SGGYYWS

SEQ ID NO: 66 - protein, 16 aa, Homo sapiens
YIFYSGSTDYNPSLKS

SEQ ID NO: 67 - protein, 10 aa, Homo sapiens
SGYSYALFDH

SEQ ID NO: 68 - protein, 5 aa, Homo sapiens
SYYLH

SEQ ID NO: 69 - protein, 17 aa, Homo sapiens
IVDPSGGSTSYDQKFQG

SEQ ID NO: 70 - protein, 9 aa, Homo sapiens
DYGDYVFDY

SEQ ID NO: 71 - protein, 7 aa, Homo sapiens
GFTFSSY

SEQ ID NO: 72 - protein, 6 aa, Homo sapiens
WYDGSN

SEQ ID NO: 73 - protein, 9 aa, Homo sapiens
GDSIISGGY

SEQ ID NO: 74 - protein, 5 aa, Homo sapiens
FYSGS

SEQ ID NO: 75 - protein, 7 aa, Homo sapiens
GYTFTSY

SEQ ID NO: 76 - protein, 6 aa, Homo sapiens
DPSGGS

SEQ ID NO: 77 - protein, 10 aa, Homo sapiens
GFTFSSYGMH

SEQ ID NO: 78 - protein, 12 aa, Homo sapiens
GDSIISGGYYWS

SEQ ID NO: 79 - protein, 10 aa, Homo sapiens
GYTFTSYYLH

SEQ ID NO: 80 - protein, 15 aa, Homo sapiens
GGGGSGGGGSGGGGS

SEQ ID NO: 81 - protein, 18 aa, Homo sapiens
GSTSGSGKPGSGEGSTKG

SEQ ID NO: 82 - DNA, 90 bp, Homo sapiens
  CDS (1)..(90): CD28T EC/spacer
cttgataatgaaaagtcaaacggaacaatcattcacgtgaagggcaagcacctctgtccgtcacccttgttccctggtccatccaagcca

SEQ ID NO: 83 - protein, 30 aa, Homo sapiens
LDNEKSNGTIIHVKGKHLCPSPLFPGPSKP

SEQ ID NO: 84 - DNA, 165 bp, Homo sapiens
  CDS (1)..(165): CD8 EC/spacer
ttcgtgcctgtttttctgcccgcgaaacccacaactacccccgcccctcggcccccaactcctgcaccaactatcgcttcccaacccctgtctctgagacctgaggcatgccgccccgcggcaggcggcgccgtgcacactagaggcctggacttcgcctgcgat

SEQ ID NO: 85 - protein, 55 aa, Homo sapiens
FVPVFLPAKPTTTPAPRPPTPAPTIASQPLSLRPEACRPAAGGAVHTRGLDFACD

SEQ ID NO: 86 - DNA, 21 bp, Homo sapiens
  CDS (1)..(21): CD8 Intracellular bit
ctctactgcaaccacagaaac

SEQ ID NO: 87 - protein, 7 aa, Homo sapiens
LYCNHRN

SEQ ID NO: 88 - DNA, 12 bp, Homo sapiens
  CDS (1)..(12): Furin cleavage site
gccaagagaagt

SEQ ID NO: 89 - protein, 4 aa, Homo sapiens
AKRS

SEQ ID NO: 90 - DNA, 54 bp, Homo sapiens
  CDS (1)..(54): T2A peptide
gagggccggggatctctccttacatgtggggacgtggaagaaaatccggggcct

SEQ ID NO: 91 - protein, 18 aa, Homo sapiens
EGRGSLLTCGDVEENPGP

SEQ ID NO: 92 - protein, 112 aa, Homo sapiens
RVKFSRSADAPAYKQGQNQLYNELNLGRREEYDVLDKRRGRDPEMGGKPRRKNPQEGLYNELQKDKMAEAYSEIGMKGERRRGKGHDGLYQGLSTATKDTYDALHMQALPPR

SEQ ID NO: 93 - protein, 47 aa, Homo sapiens
TTTPAPRPPTPAPTIASQPLSLRPEACRPAAGGAVHTRGLDFACDIY

SEQ ID NO: 94 - protein, 22 aa, Homo sapiens
IWAPLAGTCGVLLLSLVITLYC

SEQ ID NO: 95 - DNA, 60 bp, Homo sapiens
atggcactccccgtaactgctctgctgctgccgttggcattgctcctgcacgccgcacgc

SEQ ID NO: 96 - DNA, 822 bp, Homo sapiens
  CDS (1)..(822): tLNGFR
atgggtgccggcgccacgggaagggctatggatggcccgcgactgcttctcctgctgttgttgggcgtgtctctcggaggcgctaaggaggcctgtccaacgggcctctacactcactccggtgaatgttgcaaagcctgtaaccttggcgagggcgtcgcacaaccttgtggtgctaaccagacagtctgtgaaccatgcctggattcagtgacattcagcgatgttgtctcagccaccgagccttgcaagccttgtaccgaatgtgtgggccttcagtccatgtccgccccctgtgtcgaagccgatgatgcagtgtgcagatgtgcctatggatattaccaggacgaaactaccgggcggtgtgaggcctgccgggtgtgtgaagccggctctggcctcgtgttcagttgccaggataagcaaaacacagtatgtgaggagtgtccagacggaacctacagcgacgaggcgaaccacgtcgacccttgcttgccgtgcaccgtctgcgaggataccgaacgccagctgagagagtgtacgcgctgggcagacgctgagtgcgaggagatccctgggagatggatcacccggagcacacctcctgagggatcagacagtacagccccgagtacccaagaaccggaggcccctccagagcaggacctgatcgcttctacagttgctggcgtggtgacgacagtcatgggatcctcacaaccagtcgtgacgcggggcacaaccgacaatctgattcctgtctactgtagcatcttggcagccgtggtcgtgggcctggtagcctacatcgcctttaagaga

SEQ ID NO: 97 - protein, 274 aa, Homo sapiens
MGAGATGRAMDGPRLLLLLLLGVSLGGAKEACPTGLYTHSGECCKACNLGEGVAQPCGANQTVCEPCLDSVTFSDVVSATEPCKPCTECVGLQSMSAPCVEADDAVCRCAYGYYQDETTGRCEACRVCEAGSGLVFSCQDKQNTVCEECPDGTYSDEANHVDPCLPCTVCEDTERQLRECTRWADAECEEIPGRWITRSTPPEGSDSTAPSTQEPEAPPEQDLIASTVAGVVTTVMGSSQPVVTRGTTDNLIPVYCSILAAVVVGLVAYIAFKR